European Patent Specification EP 3 682 029 B1, published August 14, 2024. Title: DETECTION OF RECOMBINASE POLYMERASE AMPLIFICATION USING DUAL-HAPTEN PROBE. Applicant: ALERE SAN DIEGO INC. Application PCT/US2018/051078. The sequence listing filed with the application follows.

SEQUENCE LISTING (4 sequences)

SEQ ID NO: 1 - DNA, 49 bp, Synthliboramphus antiquus
aaatttctacttttggccagttctacaatttgttatatcacatggatgt

SEQ ID NO: 2 - DNA, 35 bp, Synthliboramphus antiquus
cagtgcccaatacacacacacaagactgggcatgg

SEQ ID NO: 3 - DNA, 35 bp, Synthliboramphus antiquus
ggtacgggtcagaacacacacacataacccgtgac

SEQ ID NO: 4 - DNA, 35 bp, Synthliboramphus antiquus
gggcatggtttctgttcccaccagctagattgcag